European Patent Application EP 4 361 179 A1, published May 1, 2024. Title: FUSED PROTEIN, FUSED PROTEIN GENERATION METHOD, ELECTRODE, REDOX DEVICE, REDOX METHOD, DISULFIDE BOND CLEAVAGE METHOD, AND ALLERGEN INACTIVATION METHOD. Applicant: Panasonic Intellectual Property Management Co., Ltd. The sequence listing filed with the application follows.

SEQUENCE LISTING (7 sequences)

SEQ ID NO: 1 - DNA, 348 bp, Artificial Sequence
  Genes encoding amino acids 32 to 146 of FTRB
atggcgaaaacggaaccgtcggagaaatcagtagagattatgaggaaattctccgagcaatatgctcgtcgctctgggacttacttctgtgttgataaaggagttacttcagtcgttattaagggtttggctgagcataaagattcatatggtgcaccgctttgcccttgcagacactatgatgataaagctgctgaggttggacaaggcttttggaattgtccgtgtgttccaatgagagagaggaaggagtgccattgtatgcttttcttaactcctgataatgatttcgctggaaaagatcagacgattacatcggatgaaataaaagaaactacagctaacatg

SEQ ID NO: 2 - DNA, 333 bp, Artificial Sequence
  Genes encoding amino acids 59 to 167 of TrxY2
atggcagcaaagaagcaaactttcaactcttttgatgatttgttgcagaactctgataaacctgtacttgtagacttctatgctacttggtgtggtccatgtcagcttatggtacctatactcaatgaagtgagtgaaacactgaaagatataattgcagttgtgaaaattgatactgagaagtacccaagtcttgctaacaaataccagattgaggctttgcccacattcatcttattcaaagacggcaaactctgggaccgtttcgagggtgccttgccagcgaaccaactcgttgagcgtattgagaattctttgcaagtgaaacagtag

SEQ ID NO: 3 - DNA, 15 bp, Artificial Sequence
  Gene encoding a linker peptide(GGGGS)1
ggcggcggcggcagc

SEQ ID NO: 4 - DNA, 30 bp, Artificial Sequence
  Gene encoding a linker peptide(GGGGS)2
ggcggcggcggcagcggcggcggcggcagc

SEQ ID NO: 5 - DNA, 45 bp, Artificial Sequence
  Gene encoding a linker peptide(GGGGS)3
ggcggcggcggcagcggcggcggcggcagcggcggcggcggcagc

SEQ ID NO: 6 - DNA, 339 bp, Artificial Sequence
  Gene encoding amino acids 73 to 184 of FTRA2
atggatattgctgtgaaatcggcggcttctgtagacgcggacgctgatctatcgtcatctacgtcgttggagacggaggaagacgagaaagcgaaggagaagattggagctagggttagggttacggttccgttgaaagtttaccatgtggttcgtgtaccggaggttgaattgatgggaatggaaggttttatcaaagattacgtcgttctttggaaaggaaagaaaatctcagctaatctgccgtttaaggtacagttcgtgaaagagatcgaaggtcgtggtcctgtcaaattcttcacgcatcttaaggaagacgagttcgagttaattgatccg

SEQ ID NO: 7 - DNA, 21 bp, Artificial Sequence
  Gene encoding histidine tag (His-Tag)
caccaccaccaccaccactga